European Patent Application EP 4 197 548 A1, published June 21, 2023. Title: ANTI-INFLAMMAATORY AND ANTI-VIRAL COMPOSITION BASED ON PLACENTA-DERIVED EXTRACELLULAR VESICLE. Applicant: TS CELL BIO CO., LTD. The sequence listing filed with the application follows.

SEQUENCE LISTING (13 sequences)

SEQ ID NO: 1 - DNA, 229 bp, Artificial Sequence
  Fig.3-A. SARS-CoV-2 3'URT sequence
caatctttaatcagtgtgtaacattagggaggacttgaaagagccaccacattttcaccgaggccacgcggagtacgatcgagtgtacagtgaacaatgctagggagagctgcctatatggaagagccctaatgtgtaaaattaattttagtagtgctatccccatgtgattttaatagcttcttaggagaatgacaaaaaaaaaaaaaaaaaaaaaaaaaaaaaaaaa

SEQ ID NO: 2 - RNA, 22 nt, Artificial Sequence
  Fig.3-B. hsa-miR-26a-5p
ucggauaggaccuaaugaacuu

SEQ ID NO: 3 - RNA, 22 nt, Artificial Sequence
  Fig.3-B. hsa-miR-92a-3p
uguccggcccuguucacguuau

SEQ ID NO: 4 - RNA, 23 nt, Artificial Sequence
  Fig.3-B. hsa-miR-181a-5p
ugaguggcugucucaacuuacaa

SEQ ID NO: 5 - RNA, 23 nt, Artificial Sequence
  Fig.3-B. hsa-miR-103a-3p
aguaucgggacauguuacgacga

SEQ ID NO: 6 - RNA, 22 nt, Artificial Sequence
  Fig.3-B. hsa-miR-92a-3p
uguccggcccuguucacguuau

SEQ ID NO: 7 - RNA, 21 nt, Artificial Sequence
  Fig.3-B. hsa-miR-23a-3p
ccuuuagggaccguuacacua

SEQ ID NO: 8 - DNA, 228 bp, Artificial Sequence
  Fig.6. 1st row; SARS-CoV-2 3'UTR sequence
caatctttaatcagtgtgtaacattagggaggacttgaaagagccaccacattttcaccgaggccacgcggagtacgatcgagtgtacagtgaacaatgctagggagagctgcctatatggaagagccctaatgtgtaaaattaattttagtagtgctatccccatgtgatttaatagcttcttaggagaatgacaaaaaaaaaaaaaaaaaaaaaaaaaaaaaaaaa

SEQ ID NO: 9 - DNA, 250 bp, Artificial Sequence
  Fig.6. 2nd row; SARS-like coronavirus_1
tgtagttaactttaatctcacatagcaatctttaatcaatgtgtaacattagggaggatttgaaagagccaccacgttctcaccgaggccacgcggagtacgatcgagggtacagtgaataatgttagggagagcagcctatatggaagagccctaatgtgtaaaattaattttagtagtgctatccccatgtgattttaatagcttcnnaaccactcgacaagaaaaaaaaaaaaaaaaaaaaaaaaaa

SEQ ID NO: 10 - DNA, 250 bp, Artificial Sequence
  Fig.6. 3rd row; SARS-like coronavirus_2
tgtagttaactttaatttcacatagcaatctttaatcaatgtgtaacattggggaggacttgaaagagccaccacgttttcaccgaggccacgcggagtacgatcgagggtacagccaataatgttagggagagcagcctatatggaagagccctaatgtgtaaaattaattttagtagtgctatccccatgtgattttaatagcttcnnaaccactcgacaagaaaaaaaaaaaaaaaaaaaaaaaaaa

SEQ ID NO: 11 - DNA, 243 bp, Artificial Sequence
  Fig.6. 4th row; SARS-like coronavirus_3
tttagttaactttaatctcacatagcaatctttaatcaatgtgtaacattagggaggacttgaaagagccaccacattttcaccgaggccacgcggagtacgatcgagggtacagtgaataatgctagggagagctgcctatatggaagagccctaatgtgtaaaattaattttagtagtgctatccccatgtgattttaatagcttcttaggagaatgacaaaaaaaaaaaaaaaaaaaaaa

SEQ ID NO: 12 - DNA, 243 bp, Artificial Sequence
  Fig.6. 5th row; SARS-like coronavirus_4
tttagttaactttaatctcacatagcaatctttaatcaatgtgtaacattagggaggacttgaaagagccaccacattttcatcgaggccacgcggagtacgatcgagggtacagtgaataatgctagggagagctgcctatatggaagagccctaatgtgtaaaattaattttagtagtgctatccccatgtgattttaatagcttcttaggagaatgacaaaaaaaaaaaaaaaaaaaaaa

SEQ ID NO: 13 - DNA, 236 bp, Artificial Sequence
  Fig.6. 6th row; SARS-like coronavirus_5
tttagttaactttaatctcacatagcaatctttaatcaatgtgtaacattagggaggacttgaaagagccaccacattttcatcgaggccacgcggagtacgatcgagggtacagtgaataatgctagggagagctgcctatatggaagagccctaatgtgtaaaattaattttagtagtgctatccccatgtgattttaatagcttcttaggagaatgacaaaaaaaaaaaaaaa